European Patent Specification EP 3 507 298 B1, published August 30, 2023. Title: DETECTING HEPATOCELLULAR CARCINOMA. Applicant: EXACT SCIENCES CORPORATION MAYO FOUNDATION FOR MEDICAL EDUCATION AND RESEARCH. The sequence listing filed with the application follows.

SEQUENCE LISTING (104 sequences)

SEQ ID NO: 1 - DNA, 17 bp, Artificial Sequence
  Synthetic
gcgcgggaggattttcg

SEQ ID NO: 2 - DNA, 18 bp, Artificial Sequence
  Synthetic
ccgccaccataaacgacc

SEQ ID NO: 3 - DNA, 21 bp, Artificial Sequence
  Synthetic
ccacggacgcgaaatcgaaat

SEQ ID NO: 4 - DNA, 21 bp, Artificial Sequence
  Synthetic
cgttcgttacgtcgttttcgt

SEQ ID NO: 5 - DNA, 17 bp, Artificial Sequence
  Synthetic
gatcgacgcgactcgac

SEQ ID NO: 6 - DNA, 21 bp, Artificial Sequence
  Synthetic
ccacggacgctcgacgtcgcc

SEQ ID NO: 7 - DNA, 17 bp, Artificial Sequence
  Synthetic
gcgggagtttggcgtag

SEQ ID NO: 8 - DNA, 21 bp, Artificial Sequence
  Synthetic
cgcgcaaataccgaataaacg

SEQ ID NO: 9 - DNA, 21 bp, Artificial Sequence
  Synthetic
ccacggacggtcggtagatcg

SEQ ID NO: 10 - DNA, 18 bp, Artificial Sequence
  Synthetic
gcgcgttgtttcgtttcg

SEQ ID NO: 11 - DNA, 20 bp, Artificial Sequence
  Synthetic
cgtcacctaccgcaaatacg

SEQ ID NO: 12 - DNA, 21 bp, Artificial Sequence
  Synthetic
ccacggacggcggataaggag

SEQ ID NO: 13 - DNA, 19 bp, Artificial Sequence
  Synthetic
agtacgtaagtagagcgcg

SEQ ID NO: 14 - DNA, 22 bp, Artificial Sequence
  Synthetic
ctaaaattaactacgccgccgt

SEQ ID NO: 15 - DNA, 21 bp, Artificial Sequence
  Synthetic
ccacggacggagaacgttcga

SEQ ID NO: 16 - DNA, 21 bp, Artificial Sequence
  Synthetic
ggcgtcgcgttttttagagaa

SEQ ID NO: 17 - DNA, 28 bp, Artificial Sequence
  Synthetic
ttccttttcgttcgtataaaatttcgtt

SEQ ID NO: 18 - DNA, 21 bp, Artificial Sequence
  Synthetic
ccacggacgatcgggttttag

SEQ ID NO: 19 - DNA, 17 bp, Artificial Sequence
  Synthetic
tgcgtatggtgggcgag

SEQ ID NO: 20 - DNA, 26 bp, Artificial Sequence
  Synthetic
cctaatttacacgtcaaccaatcgaa

SEQ ID NO: 21 - DNA, 21 bp, Artificial Sequence
  Synthetic
ccacggacggcgcgtgcgttt

SEQ ID NO: 22 - DNA, 27 bp, Artificial Sequence
  Synthetic
tttgtttttttgattaggtgtttaaga

SEQ ID NO: 23 - DNA, 21 bp, Artificial Sequence
  Synthetic
caccaacctcataaccttatc

SEQ ID NO: 24 - DNA, 21 bp, Artificial Sequence
  Synthetic
gacgcggagatagtgttgtgg

SEQ ID NO: 25 - DNA, 22 bp, Artificial Sequence
  Synthetic
gcgttttagttagatagggcgg

SEQ ID NO: 26 - DNA, 20 bp, Artificial Sequence
  Synthetic
gaaaaccccttccccgaaac

SEQ ID NO: 27 - DNA, 20 bp, Artificial Sequence
  Synthetic
cgccgaggcgcacgcctaaa

SEQ ID NO: 28 - DNA, 26 bp, Artificial Sequence
  Synthetic
agtcgtttttttaggtagtttaggcg

SEQ ID NO: 29 - DNA, 19 bp, Artificial Sequence
  Synthetic
cgacctttacaatcgccgc

SEQ ID NO: 30 - DNA, 20 bp, Artificial Sequence
  Synthetic
cgccgaggggcggtagttgt

SEQ ID NO: 31 - DNA, 16 bp, Artificial Sequence
  Synthetic
gggagcggtcgcgtag

SEQ ID NO: 32 - DNA, 28 bp, Artificial Sequence
  Synthetic
gcacctaactaaacaaaacgaactaaac

SEQ ID NO: 33 - DNA, 20 bp, Artificial Sequence
  Synthetic
cgccgaggcgcaaacgcaaa

SEQ ID NO: 34 - DNA, 17 bp, Artificial Sequence
  Synthetic
aggtggcgcgtattacg

SEQ ID NO: 35 - DNA, 20 bp, Artificial Sequence
  Synthetic
cctactaaacgcgctcaacc

SEQ ID NO: 36 - DNA, 20 bp, Artificial Sequence
  Synthetic
cgccgaggcgctcgattccc

SEQ ID NO: 37 - DNA, 19 bp, Artificial Sequence
  Synthetic
ttcgatattgggtgtcgcg

SEQ ID NO: 38 - DNA, 21 bp, Artificial Sequence
  Synthetic
cgcgaaaaccaaaaacgaaac

SEQ ID NO: 39 - DNA, 20 bp, Artificial Sequence
  Synthetic
cgccgagggaggcggggttc

SEQ ID NO: 40 - DNA, 19 bp, Artificial Sequence
  Synthetic
gcgttaatttcgcgaggta

SEQ ID NO: 41 - DNA, 28 bp, Artificial Sequence
  Synthetic
acaatactcttatatattaacgccgctc

SEQ ID NO: 42 - DNA, 20 bp, Artificial Sequence
  Synthetic
cgccgaggaggcgacggagg

SEQ ID NO: 43 - DNA, 19 bp, Artificial Sequence
  Synthetic
tttgtttcggtttttggcg

SEQ ID NO: 44 - DNA, 21 bp, Artificial Sequence
  Synthetic
accataaacgaccgaaatcga

SEQ ID NO: 45 - DNA, 21 bp, Artificial Sequence
  Synthetic
ccacggacggcgggaggattt

SEQ ID NO: 46 - DNA, 21 bp, Artificial Sequence
  Synthetic
cgttcgttacgtcgttttcgt

SEQ ID NO: 47 - DNA, 17 bp, Artificial Sequence
  Synthetic
gatcgacgcgactcgac

SEQ ID NO: 48 - DNA, 21 bp, Artificial Sequence
  Synthetic
ccacggacgctcgacgtcgcc

SEQ ID NO: 49 - DNA, 22 bp, Artificial Sequence
  Synthetic
gcgttttagttagatagggcgg

SEQ ID NO: 50 - DNA, 20 bp, Artificial Sequence
  Synthetic
gaaaaccccttccccgaaac

SEQ ID NO: 51 - DNA, 20 bp, Artificial Sequence
  Synthetic
cgccgaggcgcacgcctaaa

SEQ ID NO: 52 - DNA, 17 bp, Artificial Sequence
  Synthetic
gcgggagtttggcgtag

SEQ ID NO: 53 - DNA, 21 bp, Artificial Sequence
  Synthetic
cgcgcaaataccgaataaacg

SEQ ID NO: 54 - DNA, 21 bp, Artificial Sequence
  Synthetic
ccacggacggtcggtagatcg

SEQ ID NO: 55 - DNA, 16 bp, Artificial Sequence
  Synthetic
gggagcggtcgcgtag

SEQ ID NO: 56 - DNA, 28 bp, Artificial Sequence
  Synthetic
gcacctaactaaacaaaacgaactaaac

SEQ ID NO: 57 - DNA, 20 bp, Artificial Sequence
  Synthetic
cgccgaggcgcaaacgcaaa

SEQ ID NO: 58 - DNA, 18 bp, Artificial Sequence
  Synthetic
gcgcgttgtttcgtttcg

SEQ ID NO: 59 - DNA, 20 bp, Artificial Sequence
  Synthetic
cgtcacctaccgcaaatacg

SEQ ID NO: 60 - DNA, 21 bp, Artificial Sequence
  Synthetic
ccacggacggcggataaggag

SEQ ID NO: 61 - DNA, 19 bp, Artificial Sequence
  Synthetic
agtacgtaagtagagcgcg

SEQ ID NO: 62 - DNA, 22 bp, Artificial Sequence
  Synthetic
ctaaaattaactacgccgccgt

SEQ ID NO: 63 - DNA, 21 bp, Artificial Sequence
  Synthetic
ccacggacggagaacgttcga

SEQ ID NO: 64 - DNA, 24 bp, Artificial Sequence
  Synthetic
cgttcgttcgttattttttttcga

SEQ ID NO: 65 - DNA, 19 bp, Artificial Sequence
  Synthetic
gcccgcgaaaaccaaaaac

SEQ ID NO: 66 - DNA, 20 bp, Artificial Sequence
  Synthetic
cgccgaggcgaaactcacct

SEQ ID NO: 67 - DNA, 22 bp, Artificial Sequence
  Synthetic
gcgtttttttttagcggggtta

SEQ ID NO: 68 - DNA, 21 bp, Artificial Sequence
  Synthetic
ccgaaactaaaattctcccgc

SEQ ID NO: 69 - DNA, 20 bp, Artificial Sequence
  Synthetic
cgccgaggatgagcgtgtta

SEQ ID NO: 70 - DNA, 19 bp, Artificial Sequence
  Synthetic
cggttttcgtttgggtacg

SEQ ID NO: 71 - DNA, 17 bp, Artificial Sequence
  Synthetic
ccaacccaaaccacgcc

SEQ ID NO: 72 - DNA, 21 bp, Artificial Sequence
  Synthetic
ccacggacgcgcgccgtacga

SEQ ID NO: 73 - DNA, 16 bp, Artificial Sequence
  Synthetic
ggaggttggcggggag

SEQ ID NO: 74 - DNA, 23 bp, Artificial Sequence
  Synthetic
catatactatcgccttccgactc

SEQ ID NO: 75 - DNA, 20 bp, Artificial Sequence
  Synthetic
cgccgaggcgtaacaaaaac

SEQ ID NO: 76 - DNA, 19 bp, Artificial Sequence
  Synthetic
tcgttttaggtgagtcgcg

SEQ ID NO: 77 - DNA, 24 bp, Artificial Sequence
  Synthetic
aaataaaaccgccgaaaaaacaac

SEQ ID NO: 78 - DNA, 21 bp, Artificial Sequence
  Synthetic
ccacggacgcgctacaaacgc

SEQ ID NO: 79 - DNA, 17 bp, Artificial Sequence
  Synthetic
ggaggggtttcgttcgt

SEQ ID NO: 80 - DNA, 29 bp, Artificial Sequence
  Synthetic
ctactatcgacgctaaaaataaaacgaac

SEQ ID NO: 81 - DNA, 20 bp, Artificial Sequence
  Synthetic
cgccgaggcgcgacctaaaa

SEQ ID NO: 82 - DNA, 17 bp, Artificial Sequence
  Synthetic
aggtggcgcgtattacg

SEQ ID NO: 83 - DNA, 20 bp, Artificial Sequence
  Synthetic
cctactaaacgcgctcaacc

SEQ ID NO: 84 - DNA, 20 bp, Artificial Sequence
  Synthetic
cgccgaggcgctcgattccc

SEQ ID NO: 85 - DNA, 19 bp, Artificial Sequence
  Synthetic
gcgttaatttcgcgaggta

SEQ ID NO: 86 - DNA, 28 bp, Artificial Sequence
  Synthetic
acaatactcttatatattaacgccgctc

SEQ ID NO: 87 - DNA, 20 bp, Artificial Sequence
  Synthetic
cgccgaggaggcgacggagg

SEQ ID NO: 88 - DNA, 26 bp, Artificial Sequence
  Synthetic
agtcgtttttttaggtagtttaggcg

SEQ ID NO: 89 - DNA, 19 bp, Artificial Sequence
  Synthetic
cgacctttacaatcgccgc

SEQ ID NO: 90 - DNA, 20 bp, Artificial Sequence
  Synthetic
cgccgaggggcggtagttgt

SEQ ID NO: 91 - DNA, 21 bp, Artificial Sequence
  Synthetic
ggcgtcgcgttttttagagaa

SEQ ID NO: 92 - DNA, 27 bp, Artificial Sequence
  Synthetic
ttccttttcgttcgtataaaatttcgt

SEQ ID NO: 93 - DNA, 21 bp, Artificial Sequence
  Synthetic
ccacggacgatcgggttttag

SEQ ID NO: 94 - DNA, 20 bp, Artificial Sequence
  Synthetic
cgccgaggatcgggttttag

SEQ ID NO: 95 - DNA, 29 bp, Artificial Sequence
  Synthetic
agccggttttccggctgagactccgcgtc

SEQ ID NO: 96 - DNA, 32 bp, Artificial Sequence
  Synthetic
  misc_feature (3)..(3): modified with quencher
tctagccggttttccggctgagactccgcgtc

SEQ ID NO: 97 - DNA, 29 bp, Artificial Sequence
  Synthetic
agccggttttccggctgagacgtccgtgg

SEQ ID NO: 98 - DNA, 31 bp, Artificial Sequence
  Synthetic
  misc_feature (3)..(3): modified with quencher
tctagccgttttccggctgagacgtccgtgg

SEQ ID NO: 99 - DNA, 28 bp, Artificial Sequence
  Synthetic
agccggttttccggctgagacctcggcg

SEQ ID NO: 100 - DNA, 31 bp, Artificial Sequence
  Synthetic
  misc_feature (3)..(3): modified with quencher
tctagccggttttccggctgagacctcggcg

SEQ ID NO: 101 - DNA, 8 bp, Artificial Sequence
  Synthetic
cgccgagg

SEQ ID NO: 102 - DNA, 9 bp, Artificial Sequence
  Synthetic
gacgcggag

SEQ ID NO: 103 - DNA, 9 bp, Artificial Sequence
  Synthetic
ccacggacg

SEQ ID NO: 104 - DNA, 8 bp, Artificial Sequence
  Synthetic
gcgcgtcc